European Patent Application EP 4 772 879 A1, published July 8, 2026. Title: Screening for and development of sodium channel blockers for the treatment of pharmacoresistant neurological disorders based on a polyamine mechanism. Applicant: Rheinische Friedrich-Wilhelms-Universität Bonn. The sequence listing filed with the application follows.

SEQUENCE LISTING (2 sequences)

SEQ ID NO: 1 - RNA, 19 nt, synthetic construct
  source 1..19: mol_type = other RNA; note = SMS siRNA-set1-S1
cgacagtattttgaacaaa

SEQ ID NO: 2 - RNA, 19 nt, synthetic construct
  source 1..19: mol_type = other RNA; note = SMS siRNA-set2-S2
gattcaccttatcaaaata